European Patent Specification EP 3 737 751 B1, published August 12, 2026. Title: ADDITIONAL PHYTASE VARIANTS AND METHODS. Applicant: Fornia BioSolutions, Inc. Oo, Khin Yang, Jie Zhang, Xiyun Banerjee, Goutami Fukushima, Tatsuya Lin Hu, Eric Sawaya, Imad N. Millet, Stephen Joshua M. Zeng, Jijiao Lu, Wenhua. The sequence listing filed with the application follows.

SEQUENCE LISTING (30 sequences)

SEQ ID NO: 1 - protein, 410 aa, Artificial Sequence
  Synthetic Phytase (CL00005023 G3P)
QSEPELKLESVVIVSRHGVRAPTKATQLMQDVTPDAWPTWPVKLGWLTPRGGELVAYLGQYQRQRLVANGLLADKGCPQPGQVAIIADVDERTRKTGEAFAAGLAPDCAITVHTQADTSRPDPLFNPLKTGVCQLDPANVTDAILSRAGGSIADFTQHYQTAFRELERVLNFPQSNLCFNREKQDESCSLTQALPSELKVSADNVSLTGAVSLASMLTEIFLLQQAQGMPEPGWGRITDSHQWNTLLSLHNAQFDLLQRTPEVARSRATPLLDLIMAALTPHPPQKQAYGVTLPTSVLFIAGHDTNLANLGGALELNWTLPGQPDNTPPGGELVFERWRRLSDNSQWIQVSLVYQTLQQMRDKTPLSLNTPPGEVKLTLPGCEERNAQGMCSLAGFTQIVNEARIPACSL

SEQ ID NO: 2 - protein, 410 aa, Artificial Sequence
  Synthetic Phytase (CL00048541 G4P)
QSEPELKLESVVIVSRHGVRAPTKATQLMQDVTPDAWPTWPVKLGWLTPRGGELVAYLGQYQRQRLVANGLLADKGCPQPGQVAIIADVDERTRKTGEAFAAGLAPDCAITVHTQADTSRPDPLFNPLKTGVCQLDPANVTDAILSRAGGSIADFTQHYQTAFRELERVLNFPQSNLCFNREKQDESCSLTQALPSELKVSADNVSLTGAVSLASMLTEIFLLQQAQGMPEPGWGRITDSHQWNTLLSLHNAQFDLLQRTPEVARSRATPLLDLIKTALTPHPPQKQAYGVTLPTSVLFIAGHDTNLANLGGALGLNWTLPGQPDNTPPGGELVFERWRRLSDNSQWIQVSLVYQTLQQMRDKTPLSLNTPPGEVKLTLPGCEERNAQGMCSLAGFTQIVNEARIPACSL

SEQ ID NO: 3 - protein, 410 aa, Artificial Sequence
  Synthetic Phytase (CL00060516 G5P)
QSEPELNLESVVIVSRHGVRAPTKATQLMQDVTPRAWPTWPVKLGWLTPRGGELVAYLGQYQRQRLAANGLLADKGCPQPGQVAIIADVDERTRKTGEAFAAGLAPDCAITVHTQADTSRPDPLFNPLKTGVCQLDPANVTDAILSRAGGSIADFTQHYQTAFRELERVLNFPQSNLCFNREKQDESCSLTQALPSELKVSADNVSLTGAVSLASMLTEIFLLQQAQGMPEPGWGRIGDSHQWNTLLSLHNAQFDLLQRTPEVARSRATPLLDLIKTALTPHPPQKQAYGVTLPTSVLFIAGHDTNLANLGGALGLNWTLPGQPDNTPPGGELVFERWRRLSDNSQWIQVSLVYQTLQQMRDKIPLSLNTPPGEVKLTLPACEERNAQGMCSLAGFTQIVNEGRIPACSL

SEQ ID NO: 4 - protein, 410 aa, Artificial Sequence
  Synthetic Phytase (CL00080812 G6P)
QSEPELNLESVVIVSRHGVRAPTKATQLMQDVTPRAWPTWPVKLGWLTPRGGELVAYLGQYQRQRLAANGLLADKGCPQPGQVAIIADVDERTRKTGEAFAAGLAPDCAITVHTQADTSRPDPLFNPLKTGVCQLDPANVTDAILSRAGGSIADFTQHYQTAFRELERVLNFNQSNLCFNREKQDESCSLTQALPSELKVSADNVSLTGAVSLASMLTEIFLLQQAQGMPEPGWGRIGDSHQWNTLLSLHNAQFDLLQRTPEVARSRATPLLDLIKTALTPHPPQKQAYGVTLPTSVLFIAGHDTNLANLGGALGLNWTLPGQPDNTPPGGELVFERWRRLSDNSQWIQVSLVYQTLQQMRDKWPLSLNTPPGEVKLTLPACEERNAQGMCSLAGFTQIVNEGRIPACSL

SEQ ID NO: 5 - protein, 410 aa, Artificial Sequence
  Synthetic Phytase (CL00082400)
QSENELNLESVVIVSRHGVRAPTKATQLMQDVTPRAWPTWPVKLGWLTPRGGELVAYLGQYQRQRLAANGLLADKGCPQPGQVAIIADVDERTRKTGEAFAAGLAPDCAITVHTQADTSRADPLFNPLKTGVCQLSPANVTDAILSRAGGSIADFTQHYQTAFRELERVLNFNQSNLCFNREKQDESCSLTQALPSELKVSADNVSLTGAVSLASMLTEIFLLQQAQGMPEPGWGRIGDSHQWNTLLSLHNAQFDLLQRTPEVARSRATPLLDLIKTALTPHPPQKQAYGVTLPTSVLFIAGHDTNLANLGGALGLNWTLPGQPDNTPPGGELVFERWRRLSDNSSWIQVSLVYQTLQQMRDKWPLSLNTPPGEVKLALPACEERNAQGMCSLAGFTQIVNEGRIPACSL

SEQ ID NO: 6 - protein, 410 aa, Artificial Sequence
  Synthetic Phytase (CL00089395)
QSEPELNLESVVIVSRHGVRAPTKATQLMQDVTPRAWPTWPVKLGWLTPRGGELVAYLGQYQRQRLAANGLLADKGCPQPGQVAIIADVDERTRKTGEAFAAGLAPDCAITVHTQADTSRPDPLFNPLKTGVCQLDVANVTDAILSRAGGSIADFTQHYQTAFRELERVLNFNQSNLCFNREKQNESCSLTQALPSELKVSADNVSLTGAVSLASMLTEIFLLQQAQGMPEPGWGRIGDSHQWNTLLSLHNAQFDLLQRTPEVARSRATPLLDLIKTALTPHPPQKQAYGVTLPTSVLFIAGHDTNLANLGGALGLNWTLPGQPDNTPPGGELVFERWRRLSDNSQWIQVSLVYQTLQQMRDKWPLSLNTPPGEVKLTLPACEERNAQGMCSLAGFTQIVNEGRIPACSL

SEQ ID NO: 7 - protein, 410 aa, Artificial Sequence
  Synthetic Phytase (CL00090520)
QSENELNLESVVIVSRHGVRAPTKATQLMQDVTPNAWPTWPVKLGWLTPRGGELVAYLGQYQRQRLAANGLLADKGCPQPGQVAIIADVDERTRKTGEAFAAGLAPDCAITVHTQADTSRPDPLFNPLKTGVCQLDPANVTDAILSRAGGSIADFTQHYQTAFRELERVLNFNQSNLCFNREKQDESCSLTQALPSELKVSADNVSLTGAVSLASMLTEIFLLQQAQGMPEPGWGRIGDSHQWNTLLSLHNAQFDLLQRTPEVARSRATPLLDLIKTALTPHPPQKQAYGVTLPTSVLFIAGHDTNLANLGGALGLNWTLPGQPDNTPPGGELVFERWRRLSDNSQWIQVSLVYQTLQQMRDKWPLSLNTPPGEVKLTLPACEERNAQGMCSLAGFTQIVNEGRIPACSL

SEQ ID NO: 8 - protein, 410 aa, Artificial Sequence
  Synthetic Phytase (CL00100223)
QSENELNLESVVIVSRHGVRAPTKATQLMQDVTPNAWPTWPVKLGWLTPRGGELVAYLGQYQRQRLAANGLLADKGCPQPGQVAIIADVDERTRKTGEAFAAGLAPDCAITVHTQADTSRADPLFNPLKTGVCQLSPANVTDAILSRAGGSIADFTQHYQTAFRELERVLNFNQSNLCFNREKQDESCSLTQALPSELKVSADNVSLTGAVSLASMLTEIFLLQQAQGMPEPGWGRIGDSHQWNTLLSLHNAQFDLLQRTPEVARSRATPLLDLIKTALTPHPPQKQAYGVTLPTSVLFIAGHDTNLANLGGALGLNWTLPGQPDNTPPGGELVFERWRRLSDNSSWIQVSLVYQTLQQMRDKWPLSLNTPPGEVKLALPACEERNAQGMCSLAGFTQIVNEGRIPACSL

SEQ ID NO: 9 - protein, 410 aa, Artificial Sequence
  Synthetic Phytase (CL00102257)
QSENELNLESVVIVSRHGVRAPTKATQLMQDVTPRAWPTWPVKLGWLTPRGGELVAYLGQYQRQRLAANGLLADKGCPQPGQVAIIADVDERTRKTGEAFAAGLAPDCAITVHTQADTSRADPLFNPLKTGVCQLSPANVTDAILSRAGGSIADFTQHYQTAFRELERVLNFNQSNLCFNREKQDESCSLTQALPSELKVSADNVSLTGAVSLASMLTEIFLLQQAQGMPEPGWGRIGDSHQWNTLLSLHNAQFDLLQRTPEVARSRATPLLDLIKTALTPHPPQKQAYGVTLPTSVLFIAGHDTNLANLGGALGLNWTLPGQPDNTPPGGELVFERWRRLSDNSQWIQVSLVYQTLQQMRDKWPLSLNTPPGEVKLALPACEERNAQGMCSLAGFTQIVNEGRIPACSL

SEQ ID NO: 10 - protein, 410 aa, Artificial Sequence
  Synthetic Phytase (CL00102259)
QSENELNLESVVIVSRHGVRAPTKATQLMQDVTPNAWPTWPVKLGWLTPRGGELVAYLGQYQRQRLAANGLLADKGCPQPGQVAIIADVDERTRKTGEAFAAGLAPDCAITVHTQADTSRADPLFNPLKTGVCQLSPANVTDAILSRAGGSIADFTQHYQTAFRELERVLNFNQSNLCFNREKQDESCSLTQALPSELKVSADNVSLTGAVSLASMLTEIFLLQQAQGMPEPGWGRIGDSHQWNTLLSLHNAQFDLLQRTPEVARSRATPLLDLIKTALTPHPPQKQAYGVTLPTSVLFIAGHDTNLANLGGALGLNWTLPGQPDNTPPGGELVFERWRRLSDNSQWIQVSLVYQTLQQMRDKWPLSLNTPPGEVKLALPACEERNAQGMCSLAGFTQIVNEGRIPACSL

SEQ ID NO: 11 - protein, 410 aa, Artificial Sequence
  Synthetic Phytase (CL00071716)
QSEPELNLESVVIVSRHGVRAPTKATQLMQDVTPRAWPTWPVKLGWLTPRGGELVAYLGQYQRQRLAANGLLADKGCPQPGQVAIIADVDERTRKTGEAFAAGLAPDCAITVHTQADTSRPDPLFNPLKTGVCQLDPANVTDAILSRAGGSIADFTQHYQTAFRELERVLNFPQSNLCFNRTKQDESCSLTQALPSELKVSADNVSLTGAVSLASMLTEIFLLQQAQGMPEPGWGRINDSHQWNTLLSLHNAQFDLLQRTPEVARSRATPLLDLIKTALTPHPPQKQAYGVTLPTSVLFIAGHDTNLANLGGALGLNWTLPGQPDNTPPGGELVFERWRRLSDNSSWIQVSLVYQTLQQMRDKIPLSLNTPPGEVKLTLPACEERNAQGMCSLAGFTQIVNEGRIPACSL

SEQ ID NO: 12 - protein, 410 aa, Artificial Sequence
  Synthetic Phytase (CL00100225)
QSEPELNLESVVIVSRHGVRAPTKATQLMQDVTPRAWPTWPVKLGWLTPRGGELVAYLGQYQRQRLAANGLLADKGCPQPGQVAIIADVDERTRKTGEAFAAGLAPDCAITVHTQADTSRADPLFNPLKTGVCQLSPANVTDAILSRAGGSIADFTQHYQTAFRELERVLNFNQSNLCFNREKQDESCSLTQALPSELKVSADNVSLTGAVSLASMLTEIFLLQQAQGMPEPGWGRIGDSHQWNTLLSLHNAQFDLLQRTPEVARSRATPLLDLIKTALTPHPPQKQAYGVTLPTSVLFIAGHDTNLANLGGALGLNWTLPGQPDNTPPGGELVFERWRRLSDNSSWIQVSLVYQTLQQMRDKWPLSLNTPPGEVKLALPACEERNAQGMCSLAGFTQIVNEGRIPACSL

SEQ ID NO: 13 - protein, 410 aa, Artificial Sequence
  Synthetic Phytase (CL00102276)
QSEPELNLESVVIVSRHGVRAPTKATQLMQDVTPRAWPTWPVKLGWLTPRGGELVAYLGQYQRQRLAANGLLADKGCPQPGQVAIIADVDERTRKTGEAFAAGLAPDCAITVHTQADTSRPDPLFNPLKTGVCQLDPANVTDAILSRAGGSIADFTQHYQTAFRELERVLNFNQSNLCFNREKQDESCSLTQALPSELKVSADNVSLTGAVSLASMLTEIFLLQQAQGMPEPGWGRIGDSHQWNTLLSLHNAQFDLLQRTPEVARSRATPLLDLIKTALTPHPPQKQAYGVTLPTSVLFIAGHDTNLANLGGALGLNWTLPGQPDNTPPGGELVFERWRRLSDNSTWIQVSLVYQTLQQMRDKWPLSLNTPPGEVKLTLPACEERNAQGMCSLAGFTQIVNEGRIPACSA

SEQ ID NO: 14 - protein, 424 aa, Artificial Sequence
  Synthetic Phytase (CL00047720 Insertion Variant)
QSEPELKLESVVIVSRHGVRAPTKATQLMQDVTPDAWPTWPVKLGWLTPRGGELVAYLGQYQRQRLVANGLLADKGCPQPGQVAIIADVDERTRKTGEAFAAGLAPDCAITVHTQADTSRPDPLFNPLKTGVCQLDPANVTLAILSRAVDPANVTHAILSRAGGSIADFTQHYQTAFRELERVLNFPQSNLCFNREKQDESCSLTQALPSELKVSADNVSLTGAVSLASMLTEIFLLQQAQGMPEPGWGRITDSHQWNTLLSLHNAQFDLLQRTPEVARSRATPLLDLIMAALTPHPPQKQAYGVTLPTSVLFIAGHDTNLANLGGALELNWTLPGQPDNTPPGGELVFERWRRLSDNSQWIQVSLVYQTLQQMRDKTPLSLNTPPGEVKLTLPGCEERNAQGMCSLAGFTQIVNEARIPACSL

SEQ ID NO: 15 - protein, 14 aa, Artificial Sequence
  Synthetic Phytase (Insertion in CL00047720)
VDPANVTHAILSRA

SEQ ID NO: 16 - protein, 14 aa, Artificial Sequence
  Synthetic Phytase (Insertion in CL00047720)
PANVTLAILSRAVD

SEQ ID NO: 17 - protein, 410 aa, Artificial Sequence
  Phytase (Wild type, G1P protein)
QSEPELKLESVVIVSRHGVRAPTKATQLMQDVTPDAWPTWPVKLGWLTPRGGELIAYLGHYQRQRLVADGLLAKKGCPQPGQVAIIADVDERTRKTGEAFAAGLAPDCAITVHTQADTSSPDPLFNPLKTGVCQLDNANVTDAILSRAGGSIADFTGHRQTAFRELERVLNFPQSNLCFNREKQDESCSLTQALPSELKVSADNVSLTGAVSLASMLTEIFLLQQAQGMPEPGWGRITDSHQWNTLLSLHNAQFYLLQRTPEVARSRATPLLDLIMAALTPHPPQKQAYGVTLPTSVLFIAGHDTNLANLGGALELNWTLPGQPDNTPPGGELVFERWRRLSDNSQWIQVSLVFQTLQQMRDKTPLSLNTPPGEVKLTLAGCEERNAQGMCSLAGFTQIVNEARIPACSL

SEQ ID NO: 18 - DNA, 1230 bp, Artificial Sequence
  Synthetic Phytase (CL00048541 G4P)
cagagtgagcctgagttgaaactggaatccgttgtcatcgtctctagacatggtgttagagcaccaaccaaggccacccaacttatgcaagatgtcaccccagacgcttggccaacctggccagtcaagctgggttggttgacacctagaggtggtgagctcgttgcttacttgggtcaataccaaagacagcgtcttgttgccaacggattgttggccgataagggttgtccacaaccaggtcaagtagctattattgctgacgtcgacgaaagaacccgtaagacaggtgaagccttcgccgccggtcttgctcctgactgtgccattaccgttcacacccaagctgacacttctagaccagatccattgttcaaccctttgaagactggtgtttgccaattggacccagctaacgttactgacgctatcttgtccagagctggaggatccattgctgacttcacccaacactaccagactgccttcagagagttggaaagagttcttaacttcccacaatccaacttgtgctttaaccgtgagaagcaagacgaatcctgttccttgactcaagcattaccatctgagttgaaggtctccgccgacaacgtctctttgaccggtgctgtcagcttggcttccatgttgactgaaatctttcttctgcaacaagctcaaggtatgcctgagccaggttggggtagaatcaccgactctcaccaatggaacaccttgttgtccttgcacaacgctcaattcgacttgctgcagagaactccagaggttgctagatccagagccaccccattgttggacttgatcaagactgctttgactcctcacccacctcaaaagcaagcctacggtgttaccttgcccacttctgtcttgttcattgccggtcacgatactaacttggcaaatctcggcggtgctttgggtttgaactggactcttcctggtcaacctgataacactccaccaggtggtgagctcgttttcgaaagatggcgtagactatctgataactctcaatggattcaggtttcgttggtctaccaaactttgcagcagatgagagacaagactccactgtctttgaacacgcctccaggagaagtcaaattgaccttgcctggatgtgaagagagaaatgctcagggtatgtgttccttggctggtttcactcaaatcgttaacgaagctagaatcccagcttgttccttg

SEQ ID NO: 19 - DNA, 1230 bp, Artificial Sequence
  Synthetic Phytase (CL00060516 G5P)
cagagtgagcctgagttgaacctggaatccgttgtcatcgtctctagacatggtgttagagcaccaaccaaggccacccaacttatgcaagatgtcaccccaagagcttggccaacctggccagtcaagctgggttggttgacacctagaggtggtgagctcgttgcttacttgggtcaataccaaagacagcgtcttgctgccaacggattgttggccgataagggttgtccacaaccaggtcaagtagctattattgctgacgtcgacgaaagaacccgtaagacaggtgaagccttcgccgccggtcttgctcctgactgtgccattaccgttcacacccaagctgacacttctagaccagatccattgttcaaccctttgaagactggtgtttgccaattggacccagctaacgttactgacgctatcttgtccagagctggaggatccattgctgacttcacccaacactaccagactgccttcagagagttggaaagagttcttaacttcccacaatccaacttgtgctttaaccgtgagaagcaagacgaatcctgttccttgactcaagcattaccatctgagttgaaggtctccgccgacaacgtctctttgaccggtgctgtcagcttggcttccatgttgactgaaatctttcttctgcaacaagctcaaggtatgcctgagccaggttggggtagaatcggtgactctcaccaatggaacaccttgttgtccttgcacaacgctcaattcgacttgctgcagagaactccagaggttgctagatccagagccaccccattgttggacttgatcaagactgctttgactcctcacccacctcaaaagcaagcctacggtgttaccttgcccacttctgtcttgttcattgccggtcacgatactaacttggcaaatctcggcggtgctttgggtttgaactggactcttcctggtcaacctgataacactccaccaggtggtgagctcgttttcgaaagatggcgtagactatctgataactctcaatggattcaggtttcgttggtctaccaaactttgcagcagatgagagacaagatcccactgtctttgaacacgcctccaggagaagtcaaattgaccttgcctgcttgtgaagagagaaatgctcagggtatgtgttccttggctggtttcactcaaatcgttaacgaaggtagaatcccagcttgttccttg

SEQ ID NO: 20 - DNA, 1230 bp, Artificial Sequence
  Synthetic Phytase (CL00080812 G6P)
cagagtgagcctgagttgaacctggaatccgttgtcatcgtctctagacatggtgttagagcaccaaccaaggccacccaacttatgcaagatgtcaccccaagagcttggccaacctggccagtcaagctgggttggttgacacctagaggtggtgagctcgttgcttacttgggtcaataccaaagacagcgtcttgctgccaacggattgttggccgataagggttgtccacaaccaggtcaagtagctattattgctgacgtcgacgaaagaacccgtaagacaggtgaagccttcgccgccggtcttgctcctgactgtgccattaccgttcacacccaagctgacacttctagaccagatccattgttcaaccctttgaagactggtgtttgccaattggacccagctaacgttactgacgctatcttgtccagagctggaggatccattgctgacttcacccaacactaccagactgccttcagagagttggaaagagttcttaacttcaaccaatccaacttgtgctttaaccgtgagaagcaagacgaatcctgttccttgactcaagcattaccatctgagttgaaggtctccgccgacaacgtctctttgaccggtgctgtcagcttggcttccatgttgactgaaatctttcttctgcaacaagctcaaggtatgcctgagccaggttggggtagaatcggtgactctcaccaatggaacaccttgttgtccttgcacaacgctcaattcgacttgctgcagagaactccagaggttgctagatccagagccaccccattgttggacttgatcaagactgctttgactcctcacccacctcaaaagcaagcctacggtgttaccttgcccacttctgtcttgttcattgccggtcacgatactaacttggcaaatctcggcggtgctttgggtttgaactggactcttcctggtcaacctgataacactccaccaggtggtgagctcgttttcgaaagatggcgtagactatctgataactctcaatggattcaggtttcgttggtctaccaaactttgcagcagatgagagacaagtggccactgtctttgaacacgcctccaggagaagtcaaattgaccttgcctgcttgtgaagagagaaatgctcagggtatgtgttccttggctggtttcactcaaatcgttaacgaaggtagaatcccagcttgttccttg

SEQ ID NO: 21 - DNA, 1230 bp, Artificial Sequence
  Synthetic Phytase (CL00082400)
cagagtgagaacgagttgaacctggaatccgttgtcatcgtctctagacatggtgttagagcaccaaccaaggccacccaacttatgcaagatgtcaccccaagagcttggccaacctggccagtcaagctgggttggttgacacctagaggtggtgagctcgttgcttacttgggtcaataccaaagacagcgtcttgctgccaacggattgttggccgataagggttgtccacaaccaggtcaagtagctattattgctgacgtcgacgaaagaacccgtaagacaggtgaagccttcgccgccggtcttgctcctgactgtgccattaccgttcacacccaagctgacacttctagagctgatccattgttcaaccctttgaagactggtgtttgccaattgtctccagctaacgttactgacgctatcttgtccagagctggaggatccattgctgacttcacccaacactaccagactgccttcagagagttggaaagagttcttaacttcaaccaatccaacttgtgctttaaccgtgagaagcaagacgaatcctgttccttgactcaagcattaccatctgagttgaaggtctccgccgacaacgtctctttgaccggtgctgtcagcttggcttccatgttgactgaaatctttcttctgcaacaagctcaaggtatgcctgagccaggttggggtagaatcggtgactctcaccaatggaacaccttgttgtccttgcacaacgctcaattcgacttgctgcagagaactccagaggttgctagatccagagccaccccattgttggacttgatcaagactgctttgactcctcacccacctcaaaagcaagcctacggtgttaccttgcccacttctgtcttgttcattgccggtcacgatactaacttggcaaatctcggcggtgctttgggtttgaactggactcttcctggtcaacctgataacactccaccaggtggtgagctcgttttcgaaagatggcgtagactatctgataactcttcttggattcaggtttcgttggtctaccaaactttgcagcagatgagagacaagtggccactgtctttgaacacgcctccaggagaagtcaaattggctttgcctgcttgtgaagagagaaatgctcagggtatgtgttccttggctggtttcactcaaatcgttaacgaaggtagaatcccagcttgttccttg

SEQ ID NO: 22 - DNA, 1230 bp, Artificial Sequence
  Synthetic Phytase (CL00089395)
cagagtgagcctgagttgaacctggaatccgttgtcatcgtctctagacatggtgttagagcaccaaccaaggccacccaacttatgcaagatgtcaccccaagagcttggccaacctggccagtcaagctgggttggttgacacctagaggtggtgagctcgttgcttacttgggtcaataccaaagacagcgtcttgctgccaacggattgttggccgataagggttgtccacaaccaggtcaagtagctattattgctgacgtcgacgaaagaacccgtaagacaggtgaagccttcgccgccggtcttgctcctgactgtgccattaccgttcacacccaagctgacacttctagaccagatccattgttcaaccctttgaagactggtgtttgccaattggacgttgctaacgttactgacgctatcttgtccagagctggaggatccattgctgacttcacccaacactaccagactgccttcagagagttggaaagagttcttaacttcaaccaatccaacttgtgctttaaccgtgagaagcaaaacgaatcctgttccttgactcaagcattaccatctgagttgaaggtctccgccgacaacgtctctttgaccggtgctgtcagcttggcttccatgttgactgaaatctttcttctgcaacaagctcaaggtatgcctgagccaggttggggtagaatcggtgactctcaccaatggaacaccttgttgtccttgcacaacgctcaattcgacttgctgcagagaactccagaggttgctagatccagagccaccccattgttggacttgatcaagactgctttgactcctcacccacctcaaaagcaagcctacggtgttaccttgcccacttctgtcttgttcattgccggtcacgatactaacttggcaaatctcggcggtgctttgggtttgaactggactcttcctggtcaacctgataacactccaccaggtggtgagctcgttttcgaaagatggcgtagactatctgataactctcaatggattcaggtttcgttggtctaccaaactttgcagcagatgagagacaagtggccactgtctttgaacacgcctccaggagaagtcaaattgaccttgcctgcttgtgaagagagaaatgctcagggtatgtgttccttggctggtttcactcaaatcgttaacgaaggtagaatcccagcttgttccttg

SEQ ID NO: 23 - DNA, 1230 bp, Artificial Sequence
  Synthetic Phytase (CL00090520)
cagagtgagaacgagttgaacctggaatccgttgtcatcgtctctagacatggtgttagagcaccaaccaaggccacccaacttatgcaagatgtcaccccaaacgcttggccaacctggccagtcaagctgggttggttgacacctagaggtggtgagctcgttgcttacttgggtcaataccaaagacagcgtcttgctgccaacggattgttggccgataagggttgtccacaaccaggtcaagtagctattattgctgacgtcgacgaaagaacccgtaagacaggtgaagccttcgccgccggtcttgctcctgactgtgccattaccgttcacacccaagctgacacttctagaccagatccattgttcaaccctttgaagactggtgtttgccaattggacccagctaacgttactgacgctatcttgtccagagctggaggatccattgctgacttcacccaacactaccagactgccttcagagagttggaaagagttcttaacttcaaccaatccaacttgtgctttaaccgtgagaagcaagacgaatcctgttccttgactcaagcattaccatctgagttgaaggtctccgccgacaacgtctctttgaccggtgctgtcagcttggcttccatgttgactgaaatctttcttctgcaacaagctcaaggtatgcctgagccaggttggggtagaatcggtgactctcaccaatggaacaccttgttgtccttgcacaacgctcaattcgacttgctgcagagaactccagaggttgctagatccagagccaccccattgttggacttgatcaagactgctttgactcctcacccacctcaaaagcaagcctacggtgttaccttgcccacttctgtcttgttcattgccggtcacgatactaacttggcaaatctcggcggtgctttgggtttgaactggactcttcctggtcaacctgataacactccaccaggtggtgagctcgttttcgaaagatggcgtagactatctgataactctcaatggattcaggtttcgttggtctaccaaactttgcagcagatgagagacaagtggccactgtctttgaacacgcctccaggagaagtcaaattgaccttgcctgcttgtgaagagagaaatgctcagggtatgtgttccttggctggtttcactcaaatcgttaacgaaggtagaatcccagcttgttccttg

SEQ ID NO: 24 - DNA, 1230 bp, Artificial Sequence
  Synthetic Phytase (CL00100223)
cagagtgagaacgagttgaacctggaatccgttgtcatcgtctctagacatggtgttagagcaccaaccaaggccacccaacttatgcaagatgtcaccccaaatgcttggccaacctggccagtcaagctgggttggttgacacctagaggtggtgagctcgttgcttacttgggtcaataccaaagacagcgtcttgctgccaacggattgttggccgataagggttgtccacaaccaggtcaagtagctattattgctgacgtcgacgaaagaacccgtaagacaggtgaagccttcgccgccggtcttgctcctgactgtgccattaccgttcacacccaagctgacacttctagagctgatccattgttcaaccctttgaagactggtgtttgccaattgtctccagctaacgttactgacgctatcttgtccagagctggaggatccattgctgacttcacccaacactaccagactgccttcagagagttggaaagagttcttaacttcaaccaatccaacttgtgctttaaccgtgagaagcaagacgaatcctgttccttgactcaagcattaccatctgagttgaaggtctccgccgacaacgtctctttgaccggtgctgtcagcttggcttccatgttgactgaaatctttcttctgcaacaagctcaaggtatgcctgagccaggttggggtagaatcggtgactctcaccaatggaacaccttgttgtccttgcacaacgctcaattcgacttgctgcagagaactccagaggttgctagatccagagccaccccattgttggacttgatcaagactgctttgactcctcacccacctcaaaagcaagcctacggtgttaccttgcccacttctgtcttgttcattgccggtcacgatactaacttggcaaatctcggcggtgctttgggtttgaactggactcttcctggtcaacctgataacactccaccaggtggtgagctcgttttcgaaagatggcgtagactatctgataactcttcttggattcaggtttcgttggtctaccaaactttgcagcagatgagagacaagtggccactgtctttgaacacgcctccaggagaagtcaaattggctttgcctgcttgtgaagagagaaatgctcagggtatgtgttccttggctggtttcactcaaatcgttaacgaaggtagaatcccagcttgttccttg

SEQ ID NO: 25 - DNA, 1230 bp, Artificial Sequence
  Synthetic Phytase (CL00102257)
cagagtgagaacgagttgaacctggaatccgttgtcatcgtctctagacatggtgttagagcaccaaccaaggccacccaacttatgcaagatgtcaccccaagagcttggccaacctggccagtcaagctgggttggttgacacctagaggtggtgagctcgttgcttacttgggtcaataccaaagacagcgtcttgctgccaacggattgttggccgataagggttgtccacaaccaggtcaagtagctattattgctgacgtcgacgaaagaacccgtaagacaggtgaagccttcgccgccggtcttgctcctgactgtgccattaccgttcacacccaagctgacacttctagagctgatccattgttcaaccctttgaagactggtgtttgccaattgtctccagctaacgttactgacgctatcttgtccagagctggaggatccattgctgacttcacccaacactaccagactgccttcagagagttggaaagagttcttaacttcaaccaatccaacttgtgctttaaccgtgagaagcaagacgaatcctgttccttgactcaagcattaccatctgagttgaaggtctccgccgacaacgtctctttgaccggtgctgtcagcttggcttccatgttgactgaaatctttcttctgcaacaagctcaaggtatgcctgagccaggttggggtagaatcggtgactctcaccaatggaacaccttgttgtccttgcacaacgctcaattcgacttgctgcagagaactccagaggttgctagatccagagccaccccattgttggacttgatcaagactgctttgactcctcacccacctcaaaagcaagcctacggtgttaccttgcccacttctgtcttgttcattgccggtcacgatactaacttggcaaatctcggcggtgctttgggtttgaactggactcttcctggtcaacctgataacactccaccaggtggtgagctcgttttcgaaagatggcgtagactatctgataactctcaatggattcaggtttcgttggtctaccaaactttgcagcagatgagagacaagtggccactgtctttgaacacgcctccaggagaagtcaaattggctttgcctgcttgtgaagagagaaatgctcagggtatgtgttccttggctggtttcactcaaatcgttaacgaaggtagaatcccagcttgttccttg

SEQ ID NO: 26 - DNA, 1230 bp, Artificial Sequence
  Synthetic Phytase (CL00102259)
cagagtgagaacgagttgaacctggaatccgttgtcatcgtctctagacatggtgttagagcaccaaccaaggccacccaacttatgcaagatgtcaccccaaatgcttggccaacctggccagtcaagctgggttggttgacacctagaggtggtgagctcgttgcttacttgggtcaataccaaagacagcgtcttgctgccaacggattgttggccgataagggttgtccacaaccaggtcaagtagctattattgctgacgtcgacgaaagaacccgtaagacaggtgaagccttcgccgccggtcttgctcctgactgtgccattaccgttcacacccaagctgacacttctagagctgatccattgttcaaccctttgaagactggtgtttgccaattgtctccagctaacgttactgacgctatcttgtccagagctggaggatccattgctgacttcacccaacactaccagactgccttcagagagttggaaagagttcttaacttcaaccaatccaacttgtgctttaaccgtgagaagcaagacgaatcctgttccttgactcaagcattaccatctgagttgaaggtctccgccgacaacgtctctttgaccggtgctgtcagcttggcttccatgttgactgaaatctttcttctgcaacaagctcaaggtatgcctgagccaggttggggtagaatcggtgactctcaccaatggaacaccttgttgtccttgcacaacgctcaattcgacttgctgcagagaactccagaggttgctagatccagagccaccccattgttggacttgatcaagactgctttgactcctcacccacctcaaaagcaagcctacggtgttaccttgcccacttctgtcttgttcattgccggtcacgatactaacttggcaaatctcggcggtgctttgggtttgaactggactcttcctggtcaacctgataacactccaccaggtggtgagctcgttttcgaaagatggcgtagactatctgataactctcaatggattcaggtttcgttggtctaccaaactttgcagcagatgagagacaagtggccactgtctttgaacacgcctccaggagaagtcaaattggctttgcctgcttgtgaagagagaaatgctcagggtatgtgttccttggctggtttcactcaaatcgttaacgaaggtagaatcccagcttgttccttg

SEQ ID NO: 27 - DNA, 1230 bp, Artificial Sequence
  Synthetic Phytase (CL00071716)
cagagtgagcctgagttgaacctggaatccgttgtcatcgtctctagacatggtgttagagcaccaaccaaggccacccaacttatgcaagatgtcaccccaagagcttggccaacctggccagtcaagctgggttggttgacacctagaggtggtgagctcgttgcttacttgggtcaataccaaagacagcgtcttgctgccaacggattgttggccgataagggttgtccacaaccaggtcaagtagctattattgctgacgtcgacgaaagaacccgtaagacaggtgaagccttcgccgccggtcttgctcctgactgtgccattaccgttcacacccaagctgacacttctagaccagatccattgttcaaccctttgaagactggtgtttgccaattggacccagctaacgttactgacgctatcttgtccagagctggaggatccattgctgacttcacccaacactaccagactgccttcagagagttggaaagagttcttaacttcccacaatccaacttgtgctttaaccgtactaagcaagacgaatcctgttccttgactcaagcattaccatctgagttgaaggtctccgccgacaacgtctctttgaccggtgctgtcagcttggcttccatgttgactgaaatctttcttctgcaacaagctcaaggtatgcctgagccaggttggggtagaatcaacgactctcaccaatggaacaccttgttgtccttgcacaacgctcaattcgacttgctgcagagaactccagaggttgctagatccagagccaccccattgttggacttgatcaagactgctttgactcctcacccacctcaaaagcaagcctacggtgttaccttgcccacttctgtcttgttcattgccggtcacgatactaacttggcaaatctcggcggtgctttgggtttgaactggactcttcctggtcaacctgataacactccaccaggtggtgagctcgttttcgaaagatggcgtagactatctgataactcttcttggattcaggtttcgttggtctaccaaactttgcagcagatgagagacaagatcccactgtctttgaacacgcctccaggagaagtcaaattgaccttgcctgcttgtgaagagagaaatgctcagggtatgtgttccttggctggtttcactcaaatcgttaacgaaggtagaatcccagcttgttccttg

SEQ ID NO: 28 - DNA, 1230 bp, Artificial Sequence
  Synthetic Phytase (CL00100225)
cagagtgagcctgagttgaacctggaatccgttgtcatcgtctctagacatggtgttagagcaccaaccaaggccacccaacttatgcaagatgtcaccccaagagcttggccaacctggccagtcaagctgggttggttgacacctagaggtggtgagctcgttgcttacttgggtcaataccaaagacagcgtcttgctgccaacggattgttggccgataagggttgtccacaaccaggtcaagtagctattattgctgacgtcgacgaaagaacccgtaagacaggtgaagccttcgccgccggtcttgctcctgactgtgccattaccgttcacacccaagctgacacttctagagctgatccattgttcaaccctttgaagactggtgtttgccaattgtctccagctaacgttactgacgctatcttgtccagagctggaggatccattgctgacttcacccaacactaccagactgccttcagagagttggaaagagttcttaacttcaaccaatccaacttgtgctttaaccgtgagaagcaagacgaatcctgttccttgactcaagcattaccatctgagttgaaggtctccgccgacaacgtctctttgaccggtgctgtcagcttggcttccatgttgactgaaatctttcttctgcaacaagctcaaggtatgcctgagccaggttggggtagaatcggtgactctcaccaatggaacaccttgttgtccttgcacaacgctcaattcgacttgctgcagagaactccagaggttgctagatccagagccaccccattgttggacttgatcaagactgctttgactcctcacccacctcaaaagcaagcctacggtgttaccttgcccacttctgtcttgttcattgccggtcacgatactaacttggcaaatctcggcggtgctttgggtttgaactggactcttcctggtcaacctgataacactccaccaggtggtgagctcgttttcgaaagatggcgtagactatctgataactcttcttggattcaggtttcgttggtctaccaaactttgcagcagatgagagacaagtggccactgtctttgaacacgcctccaggagaagtcaaattggctttgcctgcttgtgaagagagaaatgctcagggtatgtgttccttggctggtttcactcaaatcgttaacgaaggtagaatcccagcttgttccttg

SEQ ID NO: 29 - DNA, 1230 bp, Artificial Sequence
  Synthetic Phytase (CL00102276)
cagagtgagcctgagttgaacctggaatccgttgtcatcgtctctagacatggtgttagagcaccaaccaaggccacccaacttatgcaagatgtcaccccaagagcttggccaacctggccagtcaagctgggttggttgacacctagaggtggtgagctcgttgcttacttgggtcaataccaaagacagcgtcttgctgccaacggattgttggccgataagggttgtccacaaccaggtcaagtagctattattgctgacgtcgacgaaagaacccgtaagacaggtgaagccttcgccgccggtcttgctcctgactgtgccattaccgttcacacccaagctgacacttctagaccagatccattgttcaaccctttgaagactggtgtttgccaattggacccagctaacgttactgacgctatcttgtccagagctggaggatccattgctgacttcacccaacactaccagactgccttcagagagttggaaagagttcttaacttcaaccaatccaacttgtgctttaaccgtgagaagcaagacgaatcctgttccttgactcaagcattaccatctgagttgaaggtctccgccgacaacgtctctttgaccggtgctgtcagcttggcttccatgttgactgaaatctttcttctgcaacaagctcaaggtatgcctgagccaggttggggtagaatcggtgactctcaccaatggaacaccttgttgtccttgcacaacgctcaattcgacttgctgcagagaactccagaggttgctagatccagagccaccccattgttggacttgatcaagactgctttgactcctcacccacctcaaaagcaagcctacggtgttaccttgcccacttctgtcttgttcattgccggtcacgatactaacttggcaaatctcggcggtgctttgggtttgaactggactcttcctggtcaacctgataacactccaccaggtggtgagctcgttttcgaaagatggcgtagactatctgataactctacttggattcaggtttcgttggtctaccaaactttgcagcagatgagagacaagtggccactgtctttgaacacgcctccaggagaagtcaaattgaccttgcctgcttgtgaagagagaaatgctcagggtatgtgttccttggctggtttcactcaaatcgttaacgaaggtagaatcccagcttgttccgct

SEQ ID NO: 30 - DNA, 1272 bp, Artificial Sequence
  Synthetic Phytase (Insertion variant)
cagagtgagcctgagttgaaactggaatccgttgtcatcgtctctagacatggtgttagagcaccaaccaaggccacccaacttatgcaagatgtcaccccagacgcttggccaacctggccagtcaagctgggttggttgacacctagaggtggtgagctcgttgcttacttgggtcaataccaaagacagcgtcttgttgccaacggattgttggccgataagggttgtccacaaccaggtcaagtagctattattgctgacgtcgacgaaagaacccgtaagacaggtgaagccttcgccgccggtcttgctcctgactgtgccattaccgttcacacccaagctgacacttctagaccagatccattgttcaaccctttgaagactggtgtttgccaattggacccagctaacgttactttggctatcttgtccagagctgtggacccagctaacgttactcatgctatcttgtccagagctggaggatccattgctgacttcacccaacactaccagactgccttcagagagttggaaagagttcttaacttcccacaatccaacttgtgctttaaccgtgagaagcaagacgaatcctgttccttgactcaagcattaccatctgagttgaaggtctccgccgacaacgtctctttgaccggtgctgtcagcttggcttccatgttgactgaaatctttcttctgcaacaagctcaaggtatgcctgagccaggttggggtagaatcaccgactctcaccaatggaacaccttgttgtccttgcacaacgctcaattcgacttgctgcagagaactccagaggttgctagatccagagccaccccattgttggacttgatcatggctgctttgactcctcacccacctcaaaagcaagcctacggtgttaccttgcccacttctgtcttgttcattgccggtcacgatactaacttggcaaatctcggcggtgctttggagttgaactggactcttcctggtcaacctgataacactccaccaggtggtgagctcgttttcgaaagatggcgtagactatctgataactctcaatggattcaggtttcgttggtctaccaaactttgcagcagatgagagacaagactccactgtctttgaacacgcctccaggagaagtcaaattgaccttgcctggatgtgaagagagaaatgctcagggtatgtgttccttggctggtttcactcaaatcgttaacgaagctagaatcccagcttgttccttg